European Patent Application EP 4 610 358 A1, published September 3, 2025. Title: FAD type Glutamate Dehydrogenase. Applicant: Kikkoman Corporation. The sequence listing filed with the application follows.

SEQUENCE LISTING (106 sequences)

SEQ ID NO: 1 - protein, 687 aa, Streptomyces sp. X-119-6
MNEMTYEQLARELLLVGPAPTNEDLKLRYLDVLIDNGLNPPGPPKRILIVGAGIAGLVAGDLLTRAGHDVTILEANANRVGGRIKTFHAKKGEPSPFADPAQYAEAGAMRLPSFHPLTLALIDKLGLKRRLFFNVDIDPQTGNQDAPVPPVFYKSFKDGKTWTNGAPSPEFKEPDKRNHTWIRTNREQVRRAQYATDPSSINEGFHLTGCETRLTVSDMVNQALEPVRDYYSVKQDDGTRVNKPFKEWLAGWADVVRDFDGYSMGRFLREYAEFSDEAVEAIGTIENMTSRLHLAFFHSFLGRSDIDPRATYWEIEGGSRMLPETLAKDLRDQIVMGQRMVRLEYYDPGRDGHHGELTGPGGPAVAIQTVPEGEPYAATQTWTGDLAIVTIPFSSLRFVKVTPPFSYKKRRAVIETHYDQATKVLLEFSRRWWEFTEADWKRELDAIAPGLYDYYQQWGEDDAEAALALPQSVRNLPTGLLGAHPSVDESRIGEEQVEYYRNSELRGGVRPATNAYGGGSTTDNPNRFMYYPSHPVPGTQGGVVLAAYSWSDDAARWDSFDDAERYGYALENLQSVHGRRIEVFYTGAGQTQSWLRDPYACGEAAVYTPHQMTAFHLDVVRPEGPVYFAGEHVSLKHAWIEGAVETAVRAAIAVNEAPVGDTGVTAAAGRRGAAAATEPMREEALTS

SEQ ID NO: 2 - DNA, 2064 bp, Streptomyces sp. X-119-6
  source 1..2064: mol_type = unassigned DNA
atgaatgaaatgacctacgagcaattggcccgcgaattgttattggttggtccggccccgacgaacgaggatcttaaattacgctatttggatgtgctgattgataacgggctgaacccgccgggtccgcctaagcgtatcttgatcgtcggggctggtattgcaggccttgttgccggagatttgttgacccgcgctgggcatgatgttactattcttgaagctaatgccaaccgtgtgggagggcgtatcaagacgttccatgcaaaaaaaggagagccatctccattcgctgatccagcgcagtacgcggaagctggggcgatgcgtcttccttcctttcacccacttaccttggcacttatcgacaagctgggcttaaaacgccgcctgttttttaatgtagatattgacccacaaactggaaatcaagatgctccagtcccaccggtcttctataagtcttttaaggacggcaagacgtggacaaatggagccccgagccctgagtttaaagagcccgataaacgtaatcacacctggatccgtacgaatcgcgaacaagtacgccgcgcccaatacgccacagacccgagctccatcaatgaaggcttccatctgacgggatgtgagacccgccttactgtctccgacatggttaaccaagcgcttgaaccggtacgcgactattattcagtcaagcaggacgatggaactcgtgtgaataagcctttcaaagaatggcttgcagggtgggccgacgtcgtgcgtgatttcgacggttattctatgggccgcttcttacgtgaatatgccgagttttcggatgaggcagtggaagcaattggcacaattgaaaacatgacctcgcgcctgcaccttgccttttttcattcgtttttgggccgttccgatatcgatccgcgcgccacttactgggagatcgagggggggtcacgcatgcttcctgaaacactggcaaaggacctgcgcgatcagatcgttatgggtcagcgcatggtacgcttagagtactatgacccgggccgcgatggccatcatggtgagcttactgggcctgggggtccggccgtggccattcagacggttccagagggagagccttacgccgcaactcaaacgtggacaggagacctggcgattgttactatcccctttagctctttacgctttgttaaagtaacgccacccttctcttataaaaagcgccgcgcggtaattgagacccattatgatcaggccaccaaagtcttacttgaatttagccgtcgttggtgggaattcacagaggcggactggaagcgtgagcttgatgctatcgccccgggtctgtacgactattatcaacagtggggtgaagacgacgccgaagcagcgcttgcactgccgcagtcagtccgcaacttgcctaccggcttgcttggggcccacccaagcgtcgacgaatcgcgtatcggagaggagcaagttgagtattatcgtaacagcgaactgcgtggcggagtgcgccctgcgaccaatgcgtacggagggggtagtacgaccgataatcctaatcgtttcatgtactatccctcccaccccgttccaggcacgcaggggggggtcgtacttgcagcatacagttggagcgatgatgcagctcgttgggattcttttgacgatgctgagcgctatggctatgcgcttgaaaacttacagtctgtccacggccgtcgtattgaggtgttctatacaggagcgggacagacccaatcatggctgcgcgatccgtacgcatgcggcgaggcagctgtctatacaccccatcaaatgaccgcgtttcacttagatgtggtgcgtcccgaggggcccgtctattttgcgggtgagcacgtttcattaaaacatgcctggatcgagggggcggtggaaacagccgttcgtgcggcgatcgctgtaaatgaagcccccgtaggtgacactggggtcacagccgctgctgggcgccgtggggcggccgccgctactgagcctatgcgcgaggaggcgttaacttcttaa

SEQ ID NO: 3 - DNA, 708 bp, synthetic construct
  misc_feature 1..708: note = StGLOD-f1
  source 1..708: mol_type = other DNA
atgaatgaaatgacctacgagcaattggcccgcgaattgttattggttggtccggccccgacgaacgaggatcttaaattacgctatttggatgtgctgattgataacgggctgaacccgccgggtccgcctaagcgtatcttgatcgtcggggctggtattgcaggccttgttgccggagatttgttgacccgcgctgggcatgatgttactattcttgaagctaatgccaaccgtgtgggagggcgtatcaagacgttccatgcaaaaaaaggagagccatctccattcgctgatccagcgcagtacgcggaagctggggcgatgcgtcttccttcctttcacccacttaccttggcacttatcgacaagctgggcttaaaacgccgcctgttttttaatgtagatattgacccacaaactggaaatcaagatgctccagtcccaccggtcttctataagtcttttaaggacggcaagacgtggacaaatggagccccgagccctgagtttaaagagcccgataaacgtaatcacacctggatccgtacgaatcgcgaacaagtacgccgcgcccaatacgccacagacccgagctccatcaatgaaggcttccatctgacgggatgtgagacccgccttactgtctccgacatggttaaccaagcgcttgaaccggtacgcgactattattcagtcaagcaggac

SEQ ID NO: 4 - DNA, 690 bp, synthetic construct
  misc_feature 1..690: note = StGLOD-f2
  source 1..690: mol_type = other DNA
tcagtcaagcaggacgatggaactcgtgtgaataagcctttcaaagaatggcttgcagggtgggccgacgtcgtgcgtgatttcgacggttattctatgggccgcttcttacgtgaatatgccgagttttcggatgaggcagtggaagcaattggcacaattgaaaacatgacctcgcgcctgcaccttgccttttttcattcgtttttgggccgttccgatatcgatccgcgcgccacttactgggagatcgagggggggtcacgcatgcttcctgaaacactggcaaaggacctgcgcgatcagatcgttatgggtcagcgcatggtacgcttagagtactatgacccgggccgcgatggccatcatggtgagcttactgggcctgggggtccggccgtggccattcagacggttccagagggagagccttacgccgcaactcaaacgtggacaggagacctggcgattgttactatcccctttagctctttacgctttgttaaagtaacgccacccttctcttataaaaagcgccgcgcggtaattgagacccattatgatcaggccaccaaagtcttacttgaatttagccgtcgttggtgggaattcacagaggcggactggaagcgtgagcttgatgctatcgccccgggtctgtacgactattatcaacagtggggtgaagac

SEQ ID NO: 5 - DNA, 696 bp, synthetic construct
  misc_feature 1..696: note = StGLOD-f3
  source 1..696: mol_type = other DNA
cagtggggtgaagacgacgccgaagcagcgcttgcactgccgcagtcagtccgcaacttgcctaccggcttgcttggggcccacccaagcgtcgacgaatcgcgtatcggagaggagcaagttgagtattatcgtaacagcgaactgcgtggcggagtgcgccctgcgaccaatgcgtacggagggggtagtacgaccgataatcctaatcgtttcatgtactatccctcccaccccgttccaggcacgcaggggggggtcgtacttgcagcatacagttggagcgatgatgcagctcgttgggattcttttgacgatgctgagcgctatggctatgcgcttgaaaacttacagtctgtccacggccgtcgtattgaggtgttctatacaggagcgggacagacccaatcatggctgcgcgatccgtacgcatgcggcgaggcagctgtctatacaccccatcaaatgaccgcgtttcacttagatgtggtgcgtcccgaggggcccgtctattttgcgggtgagcacgtttcattaaaacatgcctggatcgagggggcggtggaaacagccgttcgtgcggcgatcgctgtaaatgaagcccccgtaggtgacactggggtcacagccgctgctgggcgccgtggggcggccgccgctactgagcctatgcgcgaggaggcgttaacttcttaa

SEQ ID NO: 6 - DNA, 40 bp, synthetic construct
  misc_feature 1..40: note = primer
  source 1..40: mol_type = other DNA
ggtcatttcattcatgaattctgtttcctgtgtgaaattg

SEQ ID NO: 7 - DNA, 38 bp, synthetic construct
  misc_feature 1..38: note = primer
  source 1..38: mol_type = other DNA
gcgttaacttcttaagcttggctgttttggcggatgag

SEQ ID NO: 8 - DNA, 30 bp, synthetic construct
  misc_feature 1..30: note = primer
  source 1..30: mol_type = other DNA
gataagaccgaagcgaccaatgcgtacgga

SEQ ID NO: 9 - DNA, 30 bp, synthetic construct
  misc_feature 1..30: note = primer
  source 1..30: mol_type = other DNA
cagcttacgataatagtcgtacagacccgg

SEQ ID NO: 10 - DNA, 30 bp, synthetic construct
  misc_feature 1..30: note = primer
  source 1..30: mol_type = other DNA
gcagagccacctgcgaccaatgcgtacgga

SEQ ID NO: 11 - DNA, 30 bp, synthetic construct
  misc_feature 1..30: note = primer
  source 1..30: mol_type = other DNA
cgcatcttgataatagtcgtacagacccgg

SEQ ID NO: 12 - protein, 638 aa, synthetic construct
  REGION 1..638: note = StGLOD delta 49Ai
MNEMTYEQLARELLLVGPAPTNEDLKLRYLDVLIDNGLNPPGPPKRILIVGAGIAGLVAGDLLTRAGHDVTILEANANRVGGRIKTFHAKKGEPSPFADPAQYAEAGAMRLPSFHPLTLALIDKLGLKRRLFFNVDIDPQTGNQDAPVPPVFYKSFKDGKTWTNGAPSPEFKEPDKRNHTWIRTNREQVRRAQYATDPSSINEGFHLTGCETRLTVSDMVNQALEPVRDYYSVKQDDGTRVNKPFKEWLAGWADVVRDFDGYSMGRFLREYAEFSDEAVEAIGTIENMTSRLHLAFFHSFLGRSDIDPRATYWEIEGGSRMLPETLAKDLRDQIVMGQRMVRLEYYDPGRDGHHGELTGPGGPAVAIQTVPEGEPYAATQTWTGDLAIVTIPFSSLRFVKVTPPFSYKKRRAVIETHYDQATKVLLEFSRRWWEFTEADWKRELDAIAPGLYDYYRKLDKTEATNAYGGGSTTDNPNRFMYYPSHPVPGTQGGVVLAAYSWSDDAARWDSFDDAERYGYALENLQSVHGRRIEVFYTGAGQTQSWLRDPYACGEAAVYTPHQMTAFHLDVVRPEGPVYFAGEHVSLKHAWIEGAVETAVRAAIAVNEAPVGDTGVTAAAGRRGAAAATEPMREEALTS

SEQ ID NO: 13 - protein, 638 aa, synthetic construct
  REGION 1..638: note = StGLOD delta 49C
MNEMTYEQLARELLLVGPAPTNEDLKLRYLDVLIDNGLNPPGPPKRILIVGAGIAGLVAGDLLTRAGHDVTILEANANRVGGRIKTFHAKKGEPSPFADPAQYAEAGAMRLPSFHPLTLALIDKLGLKRRLFFNVDIDPQTGNQDAPVPPVFYKSFKDGKTWTNGAPSPEFKEPDKRNHTWIRTNREQVRRAQYATDPSSINEGFHLTGCETRLTVSDMVNQALEPVRDYYSVKQDDGTRVNKPFKEWLAGWADVVRDFDGYSMGRFLREYAEFSDEAVEAIGTIENMTSRLHLAFFHSFLGRSDIDPRATYWEIEGGSRMLPETLAKDLRDQIVMGQRMVRLEYYDPGRDGHHGELTGPGGPAVAIQTVPEGEPYAATQTWTGDLAIVTIPFSSLRFVKVTPPFSYKKRRAVIETHYDQATKVLLEFSRRWWEFTEADWKRELDAIAPGLYDYYQDAAEPPATNAYGGGSTTDNPNRFMYYPSHPVPGTQGGVVLAAYSWSDDAARWDSFDDAERYGYALENLQSVHGRRIEVFYTGAGQTQSWLRDPYACGEAAVYTPHQMTAFHLDVVRPEGPVYFAGEHVSLKHAWIEGAVETAVRAAIAVNEAPVGDTGVTAAAGRRGAAAATEPMREEALTS

SEQ ID NO: 14 - DNA, 30 bp, synthetic construct
  misc_feature 1..30: note = primer
  source 1..30: mol_type = other DNA
cgtcttgatacgccctcccacacggttggc

SEQ ID NO: 15 - DNA, 30 bp, synthetic construct
  misc_feature 1..30: note = primer
  source 1..30: mol_type = other DNA
cgtatcaagacgtaccatgcaaaaaaagga

SEQ ID NO: 16 - DNA, 30 bp, synthetic construct
  misc_feature 1..30: note = primer
  source 1..30: mol_type = other DNA
ctgcgctggatcagcgaatggagatggctc

SEQ ID NO: 17 - DNA, 30 bp, synthetic construct
  misc_feature 1..30: note = primer
  source 1..30: mol_type = other DNA
gatccagcgcagttcgcggaagctggggcg

SEQ ID NO: 18 - DNA, 30 bp, synthetic construct
  misc_feature 1..30: note = primer
  source 1..30: mol_type = other DNA
gatccagcgcagttagcggaagctggggcg

SEQ ID NO: 19 - DNA, 30 bp, synthetic construct
  misc_feature 1..30: note = primer
  source 1..30: mol_type = other DNA
gatccagcgcaggtcgcggaagctggggcg

SEQ ID NO: 20 - DNA, 30 bp, synthetic construct
  misc_feature 1..30: note = primer
  source 1..30: mol_type = other DNA
gatccagcgcagatcgcggaagctggggcg

SEQ ID NO: 21 - DNA, 30 bp, synthetic construct
  misc_feature 1..30: note = primer
  source 1..30: mol_type = other DNA
gatccagcgcagatggcggaagctggggcg

SEQ ID NO: 22 - DNA, 30 bp, synthetic construct
  misc_feature 1..30: note = primer
  source 1..30: mol_type = other DNA
aaacaggcggcgttttaagcccagcttgtc

SEQ ID NO: 23 - DNA, 30 bp, synthetic construct
  misc_feature 1..30: note = primer
  source 1..30: mol_type = other DNA
cgccgcctgttttataatgtagatattgac

SEQ ID NO: 24 - DNA, 30 bp, synthetic construct
  misc_feature 1..30: note = primer
  source 1..30: mol_type = other DNA
cgccgcctgtttttaaatgtagatattgac

SEQ ID NO: 25 - DNA, 30 bp, synthetic construct
  misc_feature 1..30: note = primer
  source 1..30: mol_type = other DNA
aaaggcaaggtgcaggcgcgaggtcatgtt

SEQ ID NO: 26 - DNA, 30 bp, synthetic construct
  misc_feature 1..30: note = primer
  source 1..30: mol_type = other DNA
caccttgcctttttacattcgtttttgggc

SEQ ID NO: 27 - DNA, 30 bp, synthetic construct
  misc_feature 1..30: note = primer
  source 1..30: mol_type = other DNA
caccttgcctttgttcattcgtttttgggc

SEQ ID NO: 28 - DNA, 30 bp, synthetic construct
  misc_feature 1..30: note = primer
  source 1..30: mol_type = other DNA
caccttgcctttattcattcgtttttgggc

SEQ ID NO: 29 - DNA, 30 bp, synthetic construct
  misc_feature 1..30: note = primer
  source 1..30: mol_type = other DNA
caccttgcctttatgcattcgtttttgggc

SEQ ID NO: 30 - DNA, 30 bp, synthetic construct
  misc_feature 1..30: note = primer
  source 1..30: mol_type = other DNA
aggctctccctctggaaccgtctgaatggc

SEQ ID NO: 31 - DNA, 30 bp, synthetic construct
  misc_feature 1..30: note = primer
  source 1..30: mol_type = other DNA
gagggagagcctttcgccgcaactcaaacg

SEQ ID NO: 32 - DNA, 30 bp, synthetic construct
  misc_feature 1..30: note = primer
  source 1..30: mol_type = other DNA
gagggagagcctttagccgcaactcaaacg

SEQ ID NO: 33 - DNA, 30 bp, synthetic construct
  misc_feature 1..30: note = primer
  source 1..30: mol_type = other DNA
gagggagagcctatcgccgcaactcaaacg

SEQ ID NO: 34 - DNA, 30 bp, synthetic construct
  misc_feature 1..30: note = primer
  source 1..30: mol_type = other DNA
gagggagagcctatggccgcaactcaaacg

SEQ ID NO: 35 - DNA, 30 bp, synthetic construct
  misc_feature 1..30: note = primer
  source 1..30: mol_type = other DNA
ggggatagtaacaatcgccaggtctcctgt

SEQ ID NO: 36 - DNA, 30 bp, synthetic construct
  misc_feature 1..30: note = primer
  source 1..30: mol_type = other DNA
gttactatccccttaagctctttacgcttt

SEQ ID NO: 37 - DNA, 30 bp, synthetic construct
  misc_feature 1..30: note = primer
  source 1..30: mol_type = other DNA
gttactatccccgttagctctttacgcttt

SEQ ID NO: 38 - DNA, 30 bp, synthetic construct
  misc_feature 1..30: note = primer
  source 1..30: mol_type = other DNA
gttactatccccattagctctttacgcttt

SEQ ID NO: 39 - DNA, 30 bp, synthetic construct
  misc_feature 1..30: note = primer
  source 1..30: mol_type = other DNA
gttactatccccatgagctctttacgcttt

SEQ ID NO: 40 - DNA, 30 bp, synthetic construct
  misc_feature 1..30: note = primer
  source 1..30: mol_type = other DNA
ttcaagtaagactttggtggcctgatcata

SEQ ID NO: 41 - DNA, 30 bp, synthetic construct
  misc_feature 1..30: note = primer
  source 1..30: mol_type = other DNA
gtcttacttgaatatagccgtcgttggtgg

SEQ ID NO: 42 - DNA, 30 bp, synthetic construct
  misc_feature 1..30: note = primer
  source 1..30: mol_type = other DNA
gtcttacttgaaatgagccgtcgttggtgg

SEQ ID NO: 43 - DNA, 30 bp, synthetic construct
  misc_feature 1..30: note = primer
  source 1..30: mol_type = other DNA
cgcattggtcgcaggtggctctgccgcatc

SEQ ID NO: 44 - DNA, 30 bp, synthetic construct
  misc_feature 1..30: note = primer
  source 1..30: mol_type = other DNA
gcgaccaatgcgttcggagggggtagtacg

SEQ ID NO: 45 - DNA, 30 bp, synthetic construct
  misc_feature 1..30: note = primer
  source 1..30: mol_type = other DNA
gcgctcagcatcgtcaaaagaatcccaacg

SEQ ID NO: 46 - DNA, 30 bp, synthetic construct
  misc_feature 1..30: note = primer
  source 1..30: mol_type = other DNA
gatgctgagcgctttggctatgcgcttgaa

SEQ ID NO: 47 - DNA, 30 bp, synthetic construct
  misc_feature 1..30: note = primer
  source 1..30: mol_type = other DNA
gatgctgagcgcttaggctatgcgcttgaa

SEQ ID NO: 48 - DNA, 30 bp, synthetic construct
  misc_feature 1..30: note = primer
  source 1..30: mol_type = other DNA
gatgctgagcgcgttggctatgcgcttgaa

SEQ ID NO: 49 - DNA, 30 bp, synthetic construct
  misc_feature 1..30: note = primer
  source 1..30: mol_type = other DNA
gatgctgagcgcatgggctatgcgcttgaa

SEQ ID NO: 50 - DNA, 30 bp, synthetic construct
  misc_feature 1..30: note = primer
  source 1..30: mol_type = other DNA
gccatagcgctcagcatcgtcaaaagaatc

SEQ ID NO: 51 - DNA, 30 bp, synthetic construct
  misc_feature 1..30: note = primer
  source 1..30: mol_type = other DNA
gagcgctatggcattgcgcttgaaaactta

SEQ ID NO: 52 - DNA, 30 bp, synthetic construct
  misc_feature 1..30: note = primer
  source 1..30: mol_type = other DNA
gagcgctatggcatggcgcttgaaaactta

SEQ ID NO: 53 - DNA, 30 bp, synthetic construct
  misc_feature 1..30: note = primer
  source 1..30: mol_type = other DNA
gaacacctcaatacgacggccgtggacaga

SEQ ID NO: 54 - DNA, 30 bp, synthetic construct
  misc_feature 1..30: note = primer
  source 1..30: mol_type = other DNA
attgaggtgttcttaacaggagcgggacag

SEQ ID NO: 55 - DNA, 30 bp, synthetic construct
  misc_feature 1..30: note = primer
  source 1..30: mol_type = other DNA
attgaggtgttcatgacaggagcgggacag

SEQ ID NO: 56 - DNA, 30 bp, synthetic construct
  misc_feature 1..30: note = primer
  source 1..30: mol_type = other DNA
cgcggtcatttgatggggtgtatagacagc

SEQ ID NO: 57 - DNA, 30 bp, synthetic construct
  misc_feature 1..30: note = primer
  source 1..30: mol_type = other DNA
caaatgaccgcgttacacttagatgtggtg

SEQ ID NO: 58 - protein, 690 aa, synthetic construct
  REGION 1..690: note = M7GLOD
MDDKTYQQLARELLLVGPEPANEDLKLRYLDVLIDNGLEPPVDRKRILIVGAGIAGLVAGHLLTRAGHDVTILEANANRVGGRIKTFHAKKGEPAPFTDPAQYAEAGAMRLPSFHPLTLALIDKLGLKRRLFFNVDIDPKTGNQGAALPPVVYKSFKDGKTWTYGKPSPEFREPDKRNHTWIRTNRTQVRRAQYVKDPSAINEGFHLTGCESRLTVSDMVNQALEPVRDYYSVLQSDGRRVNKPFKEWLDGWAGVIRDFDGFSMGRFLREYAGFSDEAVEAIGTIENMTSRLHLAFFHSFLGRSDIDPSATYWEIEGGSRQLPEALAKDLRDQIVMGQRMVRLEYYDPGRDGHHGGLAGPSGPAVAIETVPENEPSAEPQTWTADLAIVTVPFSSLRFVAVTPPFSYKKRRAVIETHYDQATKVLLEFSRRWWEFTEEDWKRELDAIAPGLYEYYQRWGEDDAEAALTVPESVRNLPTGLLGAHPSVDEQLIDDEQVEYLRNSTLRGGVRPATQVHGGGSTTDNPNRFMYYPSHAVPGSKGGVVLAAYSWSDDAARWDSFDDAERYGYALENLQSVHGRRIEVFYTGAGQTQSWLRDPYACGEAAVYTPHQMTSFHLDVVRPEGPVYFAGEHVSLKHAWIEGAVETAVRAAIAVNEAPVPYDTAAARAEAPRERAGTASATRTREKAVTS

SEQ ID NO: 59 - protein, 641 aa, synthetic construct
  REGION 1..641: note = M7GLOD delta 49C
MDDKTYQQLARELLLVGPEPANEDLKLRYLDVLIDNGLEPPVDRKRILIVGAGIAGLVAGHLLTRAGHDVTILEANANRVGGRIKTFHAKKGEPAPFTDPAQYAEAGAMRLPSFHPLTLALIDKLGLKRRLFFNVDIDPKTGNQGAALPPVVYKSFKDGKTWTYGKPSPEFREPDKRNHTWIRTNRTQVRRAQYVKDPSAINEGFHLTGCESRLTVSDMVNQALEPVRDYYSVLQSDGRRVNKPFKEWLDGWAGVIRDFDGFSMGRFLREYAGFSDEAVEAIGTIENMTSRLHLAFFHSFLGRSDIDPSATYWEIEGGSRQLPEALAKDLRDQIVMGQRMVRLEYYDPGRDGHHGGLAGPSGPAVAIETVPENEPSAEPQTWTADLAIVTVPFSSLRFVAVTPPFSYKKRRAVIETHYDQATKVLLEFSRRWWEFTEEDWKRELDAIAPGLYEYYQDAAEPPATQVHGGGSTTDNPNRFMYYPSHAVPGSKGGVVLAAYSWSDDAARWDSFDDAERYGYALENLQSVHGRRIEVFYTGAGQTQSWLRDPYACGEAAVYTPHQMTSFHLDVVRPEGPVYFAGEHVSLKHAWIEGAVETAVRAAIAVNEAPVPYDTAAARAEAPRERAGTASATRTREKAVTS

SEQ ID NO: 60 - protein, 641 aa, synthetic construct
  REGION 1..641: note = M7GLOD delta 49C-T8
MDDKTYQQLARELLLVGPEPANEDLKLRYLDVLIDNGLEPPVDRKRILIVGAGIAGLVAGHLLTRAGHDVTILEANANRVGGRIKTYHAKKGEPAPFTDPAQIAEAGAMRLPSFHPLTLALIDKLGLKRRLFYNVDIDPKTGNQGAALPPVVYKSFKDGKTWTYGKPSPEFREPDKRNHTWIRTNRTQVRRAQYVKDPSAINEGFHLTGCESRLTVSDMVNQALEPVRDYYSVLQSDGRRVNKPFKEWLDGWAGVIRDFDGFSMGRFLREYAGFSDEAVEAIGTIENMTSRLHLAFMHSFLGRSDIDPSATYWEIEGGSRQLPEALAKDLRDQIVMGQRMVRLEYYDPGRDGHHGGLAGPSGPAVAIETVPENEPSAEPQTWTADLAIVTVPLSSLRFVAVTPPFSYKKRRAVIETHYDQATKVLLEYSRRWWEFTEEDWKRELDAIAPGLYEYYQDAAEPPATQVHGGGSTTDNPNRFMYYPSHAVPGSKGGVVLAAYSWSDDAARWDSFDDAERFGYALENLQSVHGRRIEVFLTGAGQTQSWLRDPYACGEAAVYTPHQMTSFHLDVVRPEGPVYFAGEHVSLKHAWIEGAVETAVRAAIAVNEAPVPYDTAAARAEAPRERAGTASATRTREKAVTS

SEQ ID NO: 61 - DNA, 1926 bp, synthetic construct
  misc_feature 1..1926: note = M7GLOD delta 49C-T8
  source 1..1926: mol_type = other DNA
atggacgacaagacctatcagcagttagcacgcgaactgctgcttgtagggcccgagccagcgaatgaagatcttaaattgcgctatttagacgtacttattgataacgggctggagcccccagtcgatcgtaaacgtatcttaattgtgggggcagggatcgccggcctggtcgcgggacatttgttgacacgcgcgggacacgatgtcaccatcctggaggcgaatgcaaatcgcgttggaggtcgcattaagacatatcatgcaaagaaaggcgaaccggcccccttcaccgacccggctcaaattgcagaggcgggagctatgcgtttgccttcattccatcccttaacgttagcgctgattgataaattagggttgaagcgtcgcttgttctataatgttgacattgaccctaagacgggcaatcaaggtgcagcattgccgcctgtcgtttacaagagctttaaggacggtaaaacttggacgtatggtaaaccttctccggaattccgtgaaccagacaaacgtaaccacacttggattcgtaccaatcgcactcaagtacgtcgcgcccagtatgtgaaggacccgagtgcgattaacgaagggttccatttaaccgggtgcgagtcgcgtttgacagtttctgatatggtgaaccaagctttagaaccggttcgtgactactattctgtattgcagagcgacgggcgccgcgtaaataagccatttaaggagtggttagacggctgggccggtgtaatccgcgatttcgacggattctcaatgggacgttttctgcgcgagtacgctgggttttcggacgaggcggtagaagcaatcggtaccatcgagaatatgacaagtcgtttgcatttggcatttatgcacagcttcttaggtcgcagtgacattgaccccagcgcgacatattgggagattgaaggcggtagccgtcagctgcctgaggctctggcaaaagacctgcgtgatcagattgtaatgggccaacgcatggtgcgtttagagtactacgacccaggacgtgatggacaccatggaggtctggcaggaccctctggtcctgcggttgcaatcgaaactgtacccgagaacgagccaagtgcagagccgcagacgtggactgcggacctggcgattgtcactgtaccactttcgtctcttcgctttgttgcggtgactcccccattcagttataaaaaacgtcgtgcagttatcgaaactcactatgatcaggcaacaaaagtgctgttagagtattctcgtcgctggtgggagtttacagaagaggactggaagcgtgagttggacgcgattgcccccggcctgtatgaatactaccaggatgctgcagaaccgccggcaactcaagttcatggaggaggttcaacaactgacaatccaaaccgttttatgtattatccgagtcacgcggtgcctggttctaagggtggtgtggttttggccgcgtatagttggagtgacgatgcagcgcgttgggattcctttgatgacgccgaacgttttggctacgccctggaaaaccttcaatcggtccatggccgccgcatcgaggtctttttaactggagctggacaaactcagtcatggttgcgcgacccctacgcctgcggtgaggccgcagtttacacaccacatcagatgacatcttttcacttagacgtagtgcgcccggaggggccagtatactttgcgggagagcatgtctctcttaagcatgcgtggatcgagggggccgttgaaaccgcggtccgtgctgcgatcgcggttaacgaagcccccgtaccatacgacacagctgctgctcgtgcggaggcccctcgcgaacgtgccggtacagcatcagccactcgcacgcgcgagaaggccgtgacttcctaa

SEQ ID NO: 62 - DNA, 655 bp, synthetic construct
  misc_feature 1..655: note = M7GLOD delta 49C-T8-f1
  source 1..655: mol_type = other DNA
ggagatatacatatggacgacaagacctatcagcagttagcacgcgaactgctgcttgtagggcccgagccagcgaatgaagatcttaaattgcgctatttagacgtacttattgataacgggctggagcccccagtcgatcgtaaacgtatcttaattgtgggggcagggatcgccggcctggtcgcgggacatttgttgacacgcgcgggacacgatgtcaccatcctggaggcgaatgcaaatcgcgttggaggtcgcattaagacatatcatgcaaagaaaggcgaaccggcccccttcaccgacccggctcaaattgcagaggcgggagctatgcgtttgccttcattccatcccttaacgttagcgctgattgataaattagggttgaagcgtcgcttgttctataatgttgacattgaccctaagacgggcaatcaaggtgcagcattgccgcctgtcgtttacaagagctttaaggacggtaaaacttggacgtatggtaaaccttctccggaattccgtgaaccagacaaacgtaaccacacttggattcgtaccaatcgcactcaagtacgtcgcgcccagtatgtgaaggacccgagtgcgattaacgaagggttccatttaaccgggtgcgagtcgcgtttga

SEQ ID NO: 63 - DNA, 670 bp, synthetic construct
  misc_feature 1..670: note = M7GLOD delta 49C-T8-f2
  source 1..670: mol_type = other DNA
gcgagtcgcgtttgacagtttctgatatggtgaaccaagctttagaaccggttcgtgactactattctgtattgcagagcgacgggcgccgcgtaaataagccatttaaggagtggttagacggctgggccggtgtaatccgcgatttcgacggattctcaatgggacgttttctgcgcgagtacgctgggttttcggacgaggcggtagaagcaatcggtaccatcgagaatatgacaagtcgtttgcatttggcatttatgcacagcttcttaggtcgcagtgacattgaccccagcgcgacatattgggagattgaaggcggtagccgtcagctgcctgaggctctggcaaaagacctgcgtgatcagattgtaatgggccaacgcatggtgcgtttagagtactacgacccaggacgtgatggacaccatggaggtctggcaggaccctctggtcctgcggttgcaatcgaaactgtacccgagaacgagccaagtgcagagccgcagacgtggactgcggacctggcgattgtcactgtaccactttcgtctcttcgctttgttgcggtgactcccccattcagttataaaaaacgtcgtgcagttatcgaaactcactatgatcaggcaacaaaagtgctgttagagtattctcgtcgctggtg

SEQ ID NO: 64 - DNA, 655 bp, synthetic construct
  misc_feature 1..655: note = M7GLOD delta 49C-T8-f3
  source 1..655: mol_type = other DNA
ttctcgtcgctggtgggagtttacagaagaggactggaagcgtgagttggacgcgattgcccccggcctgtatgaatactaccaggatgctgcagaaccgccggcaactcaagttcatggaggaggttcaacaactgacaatccaaaccgttttatgtattatccgagtcacgcggtgcctggttctaagggtggtgtggttttggccgcgtatagttggagtgacgatgcagcgcgttgggattcctttgatgacgccgaacgttttggctacgccctggaaaaccttcaatcggtccatggccgccgcatcgaggtctttttaactggagctggacaaactcagtcatggttgcgcgacccctacgcctgcggtgaggccgcagtttacacaccacatcagatgacatcttttcacttagacgtagtgcgcccggaggggccagtatactttgcgggagagcatgtctctcttaagcatgcgtggatcgagggggccgttgaaaccgcggtccgtgctgcgatcgcggttaacgaagcccccgtaccatacgacacagctgctgctcgtgcggaggcccctcgcgaacgtgccggtacagcatcagccactcgcacgcgcgagaaggccgtgacttcctaacaaagcccgaaa

SEQ ID NO: 65 - DNA, 24 bp, synthetic construct
  misc_feature 1..24: note = primer
  source 1..24: mol_type = other DNA
catatgtatatctccttcttaaag

SEQ ID NO: 66 - DNA, 20 bp, synthetic construct
  misc_feature 1..20: note = primer
  source 1..20: mol_type = other DNA
taacaaagcccgaaaggaag

SEQ ID NO: 67 - DNA, 30 bp, synthetic construct
  misc_feature 1..30: note = primer
  source 1..30: mol_type = other DNA
ggtggtgtggttgcggccgcgtatagttgg

SEQ ID NO: 68 - DNA, 30 bp, synthetic construct
  misc_feature 1..30: note = primer
  source 1..30: mol_type = other DNA
ggtggtgtggttggtgccgcgtatagttgg

SEQ ID NO: 69 - DNA, 30 bp, synthetic construct
  misc_feature 1..30: note = primer
  source 1..30: mol_type = other DNA
ggtggtgtggttgtggccgcgtatagttgg

SEQ ID NO: 70 - DNA, 30 bp, synthetic construct
  misc_feature 1..30: note = primer
  source 1..30: mol_type = other DNA
ggtggtgtggttatggccgcgtatagttgg

SEQ ID NO: 71 - DNA, 30 bp, synthetic construct
  misc_feature 1..30: note = primer
  source 1..30: mol_type = other DNA
ggtggtgtggttaacgccgcgtatagttgg

SEQ ID NO: 72 - DNA, 30 bp, synthetic construct
  misc_feature 1..30: note = primer
  source 1..30: mol_type = other DNA
ggtggtgtggtttgcgccgcgtatagttgg

SEQ ID NO: 73 - DNA, 30 bp, synthetic construct
  misc_feature 1..30: note = primer
  source 1..30: mol_type = other DNA
ggtggtgtggtttcggccgcgtatagttgg

SEQ ID NO: 74 - DNA, 30 bp, synthetic construct
  misc_feature 1..30: note = primer
  source 1..30: mol_type = other DNA
ggtggtgtggttacggccgcgtatagttgg

SEQ ID NO: 75 - DNA, 30 bp, synthetic construct
  misc_feature 1..30: note = primer
  source 1..30: mol_type = other DNA
gcaacaaaagtgcagttagagtattctcgt

SEQ ID NO: 76 - DNA, 20 bp, synthetic construct
  misc_feature 1..20: note = primer
  source 1..20: mol_type = other DNA
aaccacaccacccttagaac

SEQ ID NO: 77 - DNA, 18 bp, synthetic construct
  misc_feature 1..18: note = primer
  source 1..18: mol_type = other DNA
cacttttgttgcctgatc

SEQ ID NO: 78 - DNA, 30 bp, synthetic construct
  misc_feature 1..30: note = primer
  source 1..30: mol_type = other DNA
gaggcgggagctgcgcgtttgccttcattc

SEQ ID NO: 79 - DNA, 30 bp, synthetic construct
  misc_feature 1..30: note = primer
  source 1..30: mol_type = other DNA
gaggcgggagcttgccgtttgccttcattc

SEQ ID NO: 80 - DNA, 30 bp, synthetic construct
  misc_feature 1..30: note = primer
  source 1..30: mol_type = other DNA
gaggcgggagctgtgcgtttgccttcattc

SEQ ID NO: 81 - DNA, 30 bp, synthetic construct
  misc_feature 1..30: note = primer
  source 1..30: mol_type = other DNA
gaggcgggagcttttcgtttgccttcattc

SEQ ID NO: 82 - DNA, 30 bp, synthetic construct
  misc_feature 1..30: note = primer
  source 1..30: mol_type = other DNA
gaggcgggagcttatcgtttgccttcattc

SEQ ID NO: 83 - DNA, 30 bp, synthetic construct
  misc_feature 1..30: note = primer
  source 1..30: mol_type = other DNA
gaggcgggagcttggcgtttgccttcattc

SEQ ID NO: 84 - DNA, 30 bp, synthetic construct
  misc_feature 1..30: note = primer
  source 1..30: mol_type = other DNA
gaggcgggagcttcgcgtttgccttcattc

SEQ ID NO: 85 - DNA, 30 bp, synthetic construct
  misc_feature 1..30: note = primer
  source 1..30: mol_type = other DNA
gaggcgggagctacgcgtttgccttcattc

SEQ ID NO: 86 - DNA, 30 bp, synthetic construct
  misc_feature 1..30: note = primer
  source 1..30: mol_type = other DNA
gaggcgggagctcagcgtttgccttcattc

SEQ ID NO: 87 - DNA, 30 bp, synthetic construct
  misc_feature 1..30: note = primer
  source 1..30: mol_type = other DNA
gaggcgggagctcatcgtttgccttcattc

SEQ ID NO: 88 - DNA, 27 bp, synthetic construct
  misc_feature 1..27: note = primer
  source 1..27: mol_type = other DNA
agctcccgcctctgcaatttgagccgg

SEQ ID NO: 89 - DNA, 30 bp, synthetic construct
  misc_feature 1..30: note = primer
  source 1..30: mol_type = other DNA
atcgaggtcttttatactggagctggacaa

SEQ ID NO: 90 - DNA, 30 bp, synthetic construct
  misc_feature 1..30: note = primer
  source 1..30: mol_type = other DNA
aaagacctcgatgcggcggccatggaccga

SEQ ID NO: 91 - protein, 641 aa, synthetic construct
  REGION 1..641: note = amino acid sequence of M7GLOD-delta-49C
MDDKTYQQLARELLLVGPEPANEDLKLRYLDVLIDNGLEPPVDRKRILIVGAGIAGLVAGHLLTRAGHDVTILEANANRVGGRIKTYHAKKGEPAPFTDPAQIAEAGAMRLPSFHPLTLALIDKLGLKRRLFYNVDIDPKTGNQGAALPPVVYKSFKDGKTWTYGKPSPEFREPDKRNHTWIRTNRTQVRRAQYVKDPSAINEGFHLTGCESRLTVSDMVNQALEPVRDYYSVLQSDGRRVNKPFKEWLDGWAGVIRDFDGFSMGRFLREYAGFSDEAVEAIGTIENMTSRLHLAFMHSFLGRSDIDPSATYWEIEGGSRQLPEALAKDLRDQIVMGQRMVRLEYYDPGRDGHHGGLAGPSGPAVAIETVPENEPSAEPQTWTADLAIVTVPLSSLRFVAVTPPFSYKKRRAVIETHYDQATKVLLEYSRRWWEFTEEDWKRELDAIAPGLYEYYQDAAEPPATQVHGGGSTTDNPNRFMYYPSHAVPGSKGGVVLAAYSWSDDAARWDSFDDAERFGYALENLQSVHGRRIEVFYTGAGQTQSWLRDPYACGEAAVYTPHQMTSFHLDVVRPEGPVYFAGEHVSLKHAWIEGAVETAVRAAIAVNEAPVPYDTAAARAEAPRERAGTASATRTREKAVTS

SEQ ID NO: 92 - DNA, 30 bp, synthetic construct
  misc_feature 1..30: note = primer
  source 1..30: mol_type = other DNA
attcgtaccaatggcactcaagtacgtcgc

SEQ ID NO: 93 - DNA, 30 bp, synthetic construct
  misc_feature 1..30: note = primer
  source 1..30: mol_type = other DNA
attcgtaccaatgcgactcaagtacgtcgc

SEQ ID NO: 94 - DNA, 30 bp, synthetic construct
  misc_feature 1..30: note = primer
  source 1..30: mol_type = other DNA
attcgtaccaattgcactcaagtacgtcgc

SEQ ID NO: 95 - DNA, 30 bp, synthetic construct
  misc_feature 1..30: note = primer
  source 1..30: mol_type = other DNA
attcgtaccaatctgactcaagtacgtcgc

SEQ ID NO: 96 - DNA, 30 bp, synthetic construct
  misc_feature 1..30: note = primer
  source 1..30: mol_type = other DNA
attcgtaccaatatgactcaagtacgtcgc

SEQ ID NO: 97 - DNA, 30 bp, synthetic construct
  misc_feature 1..30: note = primer
  source 1..30: mol_type = other DNA
attcgtaccaattttactcaagtacgtcgc

SEQ ID NO: 98 - DNA, 30 bp, synthetic construct
  misc_feature 1..30: note = primer
  source 1..30: mol_type = other DNA
attcgtaccaattatactcaagtacgtcgc

SEQ ID NO: 99 - DNA, 30 bp, synthetic construct
  misc_feature 1..30: note = primer
  source 1..30: mol_type = other DNA
attcgtaccaatagcactcaagtacgtcgc

SEQ ID NO: 100 - DNA, 30 bp, synthetic construct
  misc_feature 1..30: note = primer
  source 1..30: mol_type = other DNA
attcgtaccaataccactcaagtacgtcgc

SEQ ID NO: 101 - DNA, 30 bp, synthetic construct
  misc_feature 1..30: note = primer
  source 1..30: mol_type = other DNA
attcgtaccaataacactcaagtacgtcgc

SEQ ID NO: 102 - DNA, 30 bp, synthetic construct
  misc_feature 1..30: note = primer
  source 1..30: mol_type = other DNA
attcgtaccaatcagactcaagtacgtcgc

SEQ ID NO: 103 - DNA, 30 bp, synthetic construct
  misc_feature 1..30: note = primer
  source 1..30: mol_type = other DNA
attcgtaccaatcatactcaagtacgtcgc

SEQ ID NO: 104 - DNA, 30 bp, synthetic construct
  misc_feature 1..30: note = primer
  source 1..30: mol_type = other DNA
attcgtaccaatgatactcaagtacgtcgc

SEQ ID NO: 105 - DNA, 30 bp, synthetic construct
  misc_feature 1..30: note = primer
  source 1..30: mol_type = other DNA
attcgtaccaatgaaactcaagtacgtcgc

SEQ ID NO: 106 - DNA, 27 bp, synthetic construct
  misc_feature 1..27: note = primer
  source 1..27: mol_type = other DNA
attggtacgaatccaagtgtggttacg